European Patent Specification EP 4 211 246 B1, published July 23, 2025. Title: ADAPTORS AND METHODS FOR HIGH EFFICIENCY CONSTRUCTION OF GENETIC LIBRARIES AND GENETIC ANALYSIS. Applicant: RESOLUTION BIOSCIENCE, INC. The sequence listing filed with the application follows.

SEQUENCE LISTING (74 sequences)

SEQ ID NO: 1 - DNA, 47 bp, Artificial Sequence
  exemplary partner oligonucleotide
gtgaaaaccaggatcaactcccgtgccagtcacatctcagatgagct

SEQ ID NO: 2 - DNA, 10 bp, Artificial Sequence
  ligation-anchor region 1
acgtatgcca

SEQ ID NO: 3 - DNA, 10 bp, Artificial Sequence
  ligation-anchor region 2
ctagcgttac

SEQ ID NO: 4 - DNA, 10 bp, Artificial Sequence
  ligation-anchor region 3
gatcgacatg

SEQ ID NO: 5 - DNA, 10 bp, Artificial Sequence
  ligation-anchor region 4
tgcatcaggt

SEQ ID NO: 6 - DNA, 10 bp, Artificial Sequence
  non-ligation-anchor region 1
tggcatacgt

SEQ ID NO: 7 - DNA, 10 bp, Artificial Sequence
  non-ligation-anchor region 2
gtaacgctag

SEQ ID NO: 8 - DNA, 10 bp, Artificial Sequence
  non-ligation-anchor region 3
catgtcgatc

SEQ ID NO: 9 - DNA, 10 bp, Artificial Sequence
  non-ligation-anchor region 4
acctgatgca

SEQ ID NO: 10 - DNA, 47 bp, Artificial Sequence
  exemplary ligation strand 1
  misc_feature (34)..(36): n is any nucleotide
tgcaggaccagagaattcgaatacaaaaatcctnnnacgtatgccat

SEQ ID NO: 11 - DNA, 47 bp, Artificial Sequence
  exemplary ligation strand 2
  misc_feature (34)..(36): n is any nucleotide
tgcaggaccagagaattcgaatacaaatgatctnnnacgtatgccat

SEQ ID NO: 12 - DNA, 47 bp, Artificial Sequence
  exemplary ligation strand 3
  misc_feature (34)..(36): n is any nucleotide
tgcaggaccagagaattcgaatacaagtaatagnnnacgtatgccat

SEQ ID NO: 13 - DNA, 47 bp, Artificial Sequence
  exemplary ligation strand 4
  misc_feature (34)..(36): n is any nucleotide
tgcaggaccagagaattcgaatacacacctccgnnnacgtatgccat

SEQ ID NO: 14 - DNA, 47 bp, Artificial Sequence
  exemplary ligation strand 5
  misc_feature (34)..(36): n is any nucleotide
tgcaggaccagagaattcgaatacacgccccatnnnacgtatgccat

SEQ ID NO: 15 - DNA, 47 bp, Artificial Sequence
  exemplary ligation strand 6
  misc_feature (34)..(36): n is any nucleotide
tgcaggaccagagaattcgaatacactaccaagnnnacgtatgccat

SEQ ID NO: 16 - DNA, 47 bp, Artificial Sequence
  exemplary ligation strand 7
  misc_feature (34)..(36): n is any nucleotide
tgcaggaccagagaattcgaatacactgtcgttnnnacgtatgccat

SEQ ID NO: 17 - DNA, 47 bp, Artificial Sequence
  exemplary ligation strand 8
  misc_feature (34)..(36): n is any nucleotide
tgcaggaccagagaattcgaatacagcaaatggnnnacgtatgccat

SEQ ID NO: 18 - DNA, 47 bp, Artificial Sequence
  exemplary ligation strand 9
  misc_feature (34)..(36): n is any nucleotide
tgcaggaccagagaattcgaatacagctcgagcnnnacgtatgccat

SEQ ID NO: 19 - DNA, 47 bp, Artificial Sequence
  exemplary ligation strand 10
  misc_feature (34)..(36): n is any nucleotide
tgcaggaccagagaattcgaatacagtccacaannnacgtatgccat

SEQ ID NO: 20 - DNA, 47 bp, Artificial Sequence
  exemplary ligation strand 11
  misc_feature (34)..(36): n is any nucleotide
tgcaggaccagagaattcgaatacagttaccctnnnacgtatgccat

SEQ ID NO: 21 - DNA, 47 bp, Artificial Sequence
  exemplary ligation strand 12
  misc_feature (34)..(36): n is any nucleotide
tgcaggaccagagaattcgaatacatagttttcnnnacgtatgccat

SEQ ID NO: 22 - DNA, 47 bp, Artificial Sequence
  exemplary ligation strand 13
  misc_feature (34)..(36): n is any nucleotide
tgcaggaccagagaattcgaatacatctcagagnnnacgtatgccat

SEQ ID NO: 23 - DNA, 47 bp, Artificial Sequence
  exemplary ligation strand 14
  misc_feature (34)..(36): n is any nucleotide
tgcaggaccagagaattcgaatacatgaccttcnnnacgtatgccat

SEQ ID NO: 24 - DNA, 47 bp, Artificial Sequence
  exemplary ligation strand 15
  misc_feature (34)..(36): n is any nucleotide
tgcaggaccagagaattcgaatacattacggcannnacgtatgccat

SEQ ID NO: 25 - DNA, 47 bp, Artificial Sequence
  exemplary ligation strand 16
  misc_feature (34)..(36): n is any nucleotide
tgcaggaccagagaattcgaatacaaacaaaacnnntgcatcaggtt

SEQ ID NO: 26 - DNA, 47 bp, Artificial Sequence
  exemplary ligation strand 17
  misc_feature (34)..(36): n is any nucleotide
tgcaggaccagagaattcgaatacaacactgcannntgcatcaggtt

SEQ ID NO: 27 - DNA, 47 bp, Artificial Sequence
  exemplary ligation strand 18
  misc_feature (34)..(36): n is any nucleotide
tgcaggaccagagaattcgaatacaatcgcgatnnntgcatcaggtt

SEQ ID NO: 28 - DNA, 47 bp, Artificial Sequence
  exemplary ligation strand 19
  misc_feature (34)..(36): n is any nucleotide
tgcaggaccagagaattcgaatacaatggtggannntgcatcaggtt

SEQ ID NO: 29 - DNA, 47 bp, Artificial Sequence
  exemplary ligation strand 20
  misc_feature (34)..(36): n is any nucleotide
tgcaggaccagagaattcgaatacacaactctcnnntgcatcaggtt

SEQ ID NO: 30 - DNA, 47 bp, Artificial Sequence
  exemplary ligation strand 21
  misc_feature (34)..(36): n is any nucleotide
tgcaggaccagagaattcgaatacacgcccgaannntgcatcaggtt

SEQ ID NO: 31 - DNA, 47 bp, Artificial Sequence
  exemplary ligation strand 22
  misc_feature (34)..(36): n is any nucleotide
tgcaggaccagagaattcgaatacacgtatgacnnntgcatcaggtt

SEQ ID NO: 32 - DNA, 47 bp, Artificial Sequence
  exemplary ligation strand 23
  misc_feature (34)..(36): n is any nucleotide
tgcaggaccagagaattcgaatacagaaacgacnnntgcatcaggtt

SEQ ID NO: 33 - DNA, 47 bp, Artificial Sequence
  exemplary ligation strand 24
  misc_feature (34)..(36): n is any nucleotide
tgcaggaccagagaattcgaatacagactctgannntgcatcaggtt

SEQ ID NO: 34 - DNA, 47 bp, Artificial Sequence
  exemplary ligation strand 25
  misc_feature (34)..(36): n is any nucleotide
tgcaggaccagagaattcgaatacagtcactctnnntgcatcaggtt

SEQ ID NO: 35 - DNA, 47 bp, Artificial Sequence
  exemplary ligation strand 26
  misc_feature (34)..(36): n is any nucleotide
tgcaggaccagagaattcgaatacatactggacnnntgcatcaggtt

SEQ ID NO: 36 - DNA, 47 bp, Artificial Sequence
  exemplary ligation strand 27
  misc_feature (34)..(36): n is any nucleotide
tgcaggaccagagaattcgaatacatgcgatacnnntgcatcaggtt

SEQ ID NO: 37 - DNA, 47 bp, Artificial Sequence
  exemplary ligation strand 28
  misc_feature (34)..(36): n is any nucleotide
tgcaggaccagagaattcgaatacatgttaatgnnntgcatcaggtt

SEQ ID NO: 38 - DNA, 47 bp, Artificial Sequence
  exemplary ligation strand 29
  misc_feature (34)..(36): n is any nucleotide
tgcaggaccagagaattcgaatacattgtacttnnntgcatcaggtt

SEQ ID NO: 39 - DNA, 47 bp, Artificial Sequence
  exemplary ligation strand 30
  misc_feature (34)..(36): n is any nucleotide
tgcaggaccagagaattcgaatacatttggctcnnntgcatcaggtt

SEQ ID NO: 40 - DNA, 47 bp, Artificial Sequence
  exemplary ligation strand 31
  misc_feature (34)..(36): n is any nucleotide
tgcaggaccagagaattcgaatacaaacgcctannngatcgacatgt

SEQ ID NO: 41 - DNA, 47 bp, Artificial Sequence
  exemplary ligation strand 32
  misc_feature (34)..(36): n is any nucleotide
tgcaggaccagagaattcgaatacaaagtttcannngatcgacatgt

SEQ ID NO: 42 - DNA, 47 bp, Artificial Sequence
  exemplary ligation strand 33
  misc_feature (34)..(36): n is any nucleotide
tgcaggaccagagaattcgaatacaacagcgaannngatcgacatgt

SEQ ID NO: 43 - DNA, 47 bp, Artificial Sequence
  exemplary ligation strand 34
  misc_feature (34)..(36): n is any nucleotide
tgcaggaccagagaattcgaatacaagcgcctgnnngatcgacatgt

SEQ ID NO: 44 - DNA, 47 bp, Artificial Sequence
  exemplary ligation strand 35
  misc_feature (34)..(36): n is any nucleotide
tgcaggaccagagaattcgaatacacaacccttnnngatcgacatgt

SEQ ID NO: 45 - DNA, 47 bp, Artificial Sequence
  exemplary ligation strand 36
  misc_feature (34)..(36): n is any nucleotide
tgcaggaccagagaattcgaatacacagaataannngatcgacatgt

SEQ ID NO: 46 - DNA, 47 bp, Artificial Sequence
  exemplary ligation strand 37
  misc_feature (34)..(36): n is any nucleotide
tgcaggaccagagaattcgaatacacggacaccnnngatcgacatgt

SEQ ID NO: 47 - DNA, 47 bp, Artificial Sequence
  exemplary ligation strand 38
  misc_feature (34)..(36): n is any nucleotide
tgcaggaccagagaattcgaatacagcctattcnnngatcgacatgt

SEQ ID NO: 48 - DNA, 47 bp, Artificial Sequence
  exemplary ligation strand 39
  misc_feature (34)..(36): n is any nucleotide
tgcaggaccagagaattcgaatacagcgtccagnnngatcgacatgt

SEQ ID NO: 49 - DNA, 47 bp, Artificial Sequence
  exemplary ligation strand 40
  misc_feature (34)..(36): n is any nucleotide
tgcaggaccagagaattcgaatacaggtacaagnnngatcgacatgt

SEQ ID NO: 50 - DNA, 47 bp, Artificial Sequence
  exemplary ligation strand 41
  misc_feature (34)..(36): n is any nucleotide
tgcaggaccagagaattcgaatacataaccctcnnngatcgacatgt

SEQ ID NO: 51 - DNA, 47 bp, Artificial Sequence
  exemplary ligation strand 42
  misc_feature (34)..(36): n is any nucleotide
tgcaggaccagagaattcgaatacataggagtgnnngatcgacatgt

SEQ ID NO: 52 - DNA, 47 bp, Artificial Sequence
  exemplary ligation strand 43
  misc_feature (34)..(36): n is any nucleotide
tgcaggaccagagaattcgaatacatccgcattnnngatcgacatgt

SEQ ID NO: 53 - DNA, 47 bp, Artificial Sequence
  exemplary ligation strand 44
  misc_feature (34)..(36): n is any nucleotide
tgcaggaccagagaattcgaatacatgcgtcaannngatcgacatgt

SEQ ID NO: 54 - DNA, 47 bp, Artificial Sequence
  exemplary ligation strand 45
  misc_feature (34)..(36): n is any nucleotide
tgcaggaccagagaattcgaatacattggtaatnnngatcgacatgt

SEQ ID NO: 55 - DNA, 47 bp, Artificial Sequence
  exemplary ligation strand 46
  misc_feature (34)..(36): n is any nucleotide
tgcaggaccagagaattcgaatacaaatagcttnnnctagcgttact

SEQ ID NO: 56 - DNA, 47 bp, Artificial Sequence
  exemplary ligation strand 47
  misc_feature (34)..(36): n is any nucleotide
tgcaggaccagagaattcgaatacaagagagagnnnctagcgttact

SEQ ID NO: 57 - DNA, 47 bp, Artificial Sequence
  exemplary ligation strand 48
  misc_feature (34)..(36): n is any nucleotide
tgcaggaccagagaattcgaatacacaacctgannnctagcgttact

SEQ ID NO: 58 - DNA, 47 bp, Artificial Sequence
  exemplary ligation strand 49
  misc_feature (34)..(36): n is any nucleotide
tgcaggaccagagaattcgaatacacatatggcnnnctagcgttact

SEQ ID NO: 59 - DNA, 47 bp, Artificial Sequence
  exemplary ligation strand 50
  misc_feature (34)..(36): n is any nucleotide
tgcaggaccagagaattcgaatacaccatatccnnnctagcgttact

SEQ ID NO: 60 - DNA, 47 bp, Artificial Sequence
  exemplary ligation strand 51
  misc_feature (34)..(36): n is any nucleotide
tgcaggaccagagaattcgaatacacgaggtccnnnctagcgttact

SEQ ID NO: 61 - DNA, 47 bp, Artificial Sequence
  exemplary ligation strand 52
  misc_feature (34)..(36): n is any nucleotide
tgcaggaccagagaattcgaatacacgtcaatgnnnctagcgttact

SEQ ID NO: 62 - DNA, 47 bp, Artificial Sequence
  exemplary ligation strand 53
  misc_feature (34)..(36): n is any nucleotide
tgcaggaccagagaattcgaatacacttatcatnnnctagcgttact

SEQ ID NO: 63 - DNA, 47 bp, Artificial Sequence
  exemplary ligation strand 54
  misc_feature (34)..(36): n is any nucleotide
tgcaggaccagagaattcgaatacagcattgacnnnctagcgttact

SEQ ID NO: 64 - DNA, 47 bp, Artificial Sequence
  exemplary ligation strand 55
  misc_feature (34)..(36): n is any nucleotide
tgcaggaccagagaattcgaatacaggaggtatnnnctagcgttact

SEQ ID NO: 65 - DNA, 47 bp, Artificial Sequence
  exemplary ligation strand 56
  misc_feature (34)..(36): n is any nucleotide
tgcaggaccagagaattcgaatacataacagttnnnctagcgttact

SEQ ID NO: 66 - DNA, 47 bp, Artificial Sequence
  exemplary ligation strand 57
  misc_feature (34)..(36): n is any nucleotide
tgcaggaccagagaattcgaatacatcgaacacnnnctagcgttact

SEQ ID NO: 67 - DNA, 47 bp, Artificial Sequence
  exemplary ligation strand 58
  misc_feature (34)..(36): n is any nucleotide
tgcaggaccagagaattcgaatacatgcataatnnnctagcgttact

SEQ ID NO: 68 - DNA, 47 bp, Artificial Sequence
  exemplary ligation strand 59
  misc_feature (34)..(36): n is any nucleotide
tgcaggaccagagaattcgaatacatgtcataannnctagcgttact

SEQ ID NO: 69 - DNA, 47 bp, Artificial Sequence
  exemplary ligation strand 60
  misc_feature (34)..(36): n is any nucleotide
tgcaggaccagagaattcgaatacattgcgcggnnnctagcgttact

SEQ ID NO: 70 - DNA, 25 bp, Artificial Sequence
  single amplification primer
tgcaggaccagagaattcgaataca

SEQ ID NO: 71 - DNA, 58 bp, Artificial Sequence
  Forward Primer
aatgatacggcgaccaccgagatctacacgtcatgcaggaccagagaattcgaataca

SEQ ID NO: 72 - DNA, 57 bp, Artificial Sequence
  Reverse Primer
caagcagaagacggcatacgagatgtgactggcacgggagttgatcctggttttcac

SEQ ID NO: 73 - DNA, 56 bp, Artificial Sequence
  Forward Seq Primer
caagcagaagacggcatacgagatgtgactggcacgggaccagagaattcgaatac

SEQ ID NO: 74 - DNA, 33 bp, Artificial Sequence
  Reverse Seq Primer 62
gtgactggcacgggaccagagaattcgaataca